European Patent Application EP 4 148 120 A1, published March 15, 2023. Title: RECOMBINANT STRAIN PRODUCING L-LYSINE AND CONSTRUCTION METHODS THEREFOR AND USE THEREOF. Applicant: HEILONGJIANG EPPEN BIOTECH CO., LTD. Application 20939893.2. The sequence listing filed with the application follows.

SEQUENCE LISTING (36 sequences)

SEQ ID NO: 1 - DNA, 1035 bp, Corynebacterium glutamicum
atggcatttgcagacattgtgcgcagcgtcgaaaaccgcaccaacgcagcgaccctcaactggtccatcaaaaatggctggaagcccgaagtcaccggattttccgggtacggctccgggcgtcgagtgcgcgtccttgcgcgcgtgctcatgtccaaccccgaaaatttgcttgtcgacgccccctcccaatcaattacccaacaagcacagcgcggttggcgccagttcttcaccatccaagtgcccaacctgccagtaactgtcaccgttggtgggaaaacagttacctcatccaccaacgacaacggctacgttgacctcctggtggaagaccacaaccttgaccccggctggcacaccatccagatccaagccgaaggttccacccccgccgaagcccgcgtcctcatcgtggaaaacaccgcccgaatcggactcatctccgacatcgacgacaccatcatggtcacctggcttccccgagcactcctcgccgcatggaactcgtgggttttgcacaccaaaacccgaaaaccagtccccggaatgaaccgcttctacgaagaactcctcaaagaccaccccgacgcacccgtgttctacctctccaccggcgcatggaacacctttgaaaccctccaagagttcatcaacaaacacgcactccccgacggccccatgctgctcaccgactggggaccaacccccacaggactattccgctcaggtcaagagcacaagaaagtccaactgcgcaacctgtttatcgaataccccgacatgaaatggatcctcgtcggcgacgatggccaacacgatcccctcatctacggcgaagcagtcgaagaacaccccaaccgcatcgcaggcgttgcaatccgtgagctctcccccggcgaacatgtgctctcccacggaacaactgcgtcactgtccaccatcacgaccaacgggggccaaggagtcccagtagttcacggccgcgatggatatgagttgctgcagcgctacgagacgaagccgttcgcctga

SEQ ID NO: 2 - DNA, 1035 bp, Artificial Sequence
  Artificial Sequence
atggcatttgcagacattgtgcgcagcgtcgaaaaccgcaccaacgcagcgaccctcaactggtccatcaaaaatggctggaagcccgaagtcaccggattttccgggtacggctccgggcgtcgagtgcgcgtccttgcgcgcgtgctcatgtccaaccccgaaaatttgcttgtcgacgccccctcccaatcaattacccaacaagcacagcgcggttggcgccagttcttcaccatccaagtgcccaacctgccagtaactgtcaccgttggtgggaaaacagttacctcatccaccaacgacaacggctacgttgacctcctggtggaagaccacaaccttgaccccggctggcacaccatccagatccaagccgaaggttccacccccgccgaagcccgcgtcctcatcgtggaaaacaccgcccgaatcggactcatctccgacatcgacgacaccatcatggtcacctggcttccccgagcactcctcgccgcatggaactcgtgggttttgcacaccaacacccgaaaaccagtccccggaatgaaccgcttctacgaagaactcctcaaagaccaccccgacgcacccgtgttctacctctccaccggcgcatggaacacctttgaaaccctccaagagttcatcaacaaacacgcactccccgacggccccatgctgctcaccgactggggaccaacccccacaggactattccgctcaggtcaagagcacaagaaagtccaactgcgcaacctgtttatcgaataccccgacatgaaatggatcctcgtcggcgacgatggccaacacgatcccctcatctacggcgaagcagtcgaagaacaccccaaccgcatcgcaggcgttgcaatccgtgagctctcccccggcgaacatgtgctctcccacggaacaactgcgtcactgtccaccatcacgaccaacgggggccaaggagtcccagtagttcacggccgcgatggatatgagttgctgcagcgctacgagacgaagccgttcgcctga

SEQ ID NO: 3 - protein, 344 aa, Corynebacterium glutamicum
MAFADIVRSVENRTNAATLNWSIKNGWKPEVTGFSGYGSGRRVRVLARVLMSNPENLLVDAPSQSITQQAQRGWRQFFTIQVPNLPVTVTVGGKTVTSSTNDNGYVDLLVEDHNLDPGWHTIQIQAEGSTPAEARVLIVENTARIGLISDIDDTIMVTWLPRALLAAWNSWVLHTKTRKPVPGMNRFYEELLKDHPDAPVFYLSTGAWNTFETLQEFINKHALPDGPMLLTDWGPTPTGLFRSGQEHKKVQLRNLFIEYPDMKWILVGDDGQHDPLIYGEAVEEHPNRIAGVAIRELSPGEHVLSHGTTASLSTITTNGGQGVPVVHGRDGYELLQRYETKPFA

SEQ ID NO: 4 - protein, 344 aa, Artificial Sequence
  Artificial Sequence
MAFADIVRSVENRTNAATLNWSIKNGWKPEVTGFSGYGSGRRVRVLARVLMSNPENLLVDAPSQSITQQAQRGWRQFFTIQVPNLPVTVTVGGKTVTSSTNDNGYVDLLVEDHNLDPGWHTIQIQAEGSTPAEARVLIVENTARIGLISDIDDTIMVTWLPRALLAAWNSWVLHTNTRKPVPGMNRFYEELLKDHPDAPVFYLSTGAWNTFETLQEFINKHALPDGPMLLTDWGPTPTGLFRSGQEHKKVQLRNLFIEYPDMKWILVGDDGQHDPLIYGEAVEEHPNRIAGVAIRELSPGEHVLSHGTTASLSTITTNGGQGVPVVHGRDGYELLQRYETKPFA

SEQ ID NO: 5 - DNA, 56 bp, Artificial Sequence
  Artificial Sequence
cagtgccaagcttgcatgcctgcaggtcgactctagcggcgaccgcatggacaccg

SEQ ID NO: 6 - DNA, 30 bp, Artificial Sequence
  Artificial Sequence
ccggggactggttttcgggtgttggtgtgc

SEQ ID NO: 7 - DNA, 30 bp, Artificial Sequence
  Artificial Sequence
gcacaccaacacccgaaaaccagtccccgg

SEQ ID NO: 8 - DNA, 58 bp, Artificial Sequence
  Artificial Sequence
cagctatgaccatgattacgaattcgagctcggtaccccgaggtctctcagaatcggt

SEQ ID NO: 9 - DNA, 18 bp, Artificial Sequence
  Artificial Sequence
gaaaacaccgcccgaatc

SEQ ID NO: 10 - DNA, 20 bp, Artificial Sequence
  Artificial Sequence
ggagtgcgtgtttgttgatg

SEQ ID NO: 11 - DNA, 55 bp, Artificial Sequence
  Artificial Sequence
cagtgccaagcttgcatgcctgcaggtcgactctagaatgcgttctggactgagg

SEQ ID NO: 12 - DNA, 54 bp, Artificial Sequence
  Artificial Sequence
aacaccattgtccctgttttgggcgaaattttcccggtgcaccgagaacagatg

SEQ ID NO: 13 - DNA, 60 bp, Artificial Sequence
  Artificial Sequence
cgggaaaatttcgcccaaaacagggacaatggtgttatggcatttgcagacattgtgcgc

SEQ ID NO: 14 - DNA, 45 bp, Artificial Sequence
  Artificial Sequence
cttgatttaattgcgccatctcaggcgaacggcttcgtctcgtag

SEQ ID NO: 15 - DNA, 45 bp, Artificial Sequence
  Artificial Sequence
ctacgagacgaagccgttcgcctgagatggcgcaattaaatcaag

SEQ ID NO: 16 - DNA, 60 bp, Artificial Sequence
  Artificial Sequence
cagctatgaccatgattacgaattcgagctcggtacccgctatgacaccttcaacggatc

SEQ ID NO: 17 - DNA, 19 bp, Artificial Sequence
  Artificial Sequence
tccaaggaagatacacgcc

SEQ ID NO: 18 - DNA, 21 bp, Artificial Sequence
  Artificial Sequence
cctgagcggaatagtcctgtg

SEQ ID NO: 19 - DNA, 19 bp, Artificial Sequence
  Artificial Sequence
acgcacccgtgttctacct

SEQ ID NO: 20 - DNA, 18 bp, Artificial Sequence
  Artificial Sequence
cgttggaatcttgcgttg

SEQ ID NO: 21 - DNA, 59 bp, Artificial Sequence
  Artificial Sequence
gcttgcatgcctgcaggtcgactctagaggatcccccgggaaaatttcgcccaaaacag

SEQ ID NO: 22 - DNA, 59 bp, Artificial Sequence
  Artificial Sequence
atcaggctgaaaatcttctctcatccgccaaaactcaggcgaacggcttcgtctcgtag

SEQ ID NO: 23 - DNA, 55 bp, Artificial Sequence
  Artificial Sequence
cagtgccaagcttgcatgcctgcaggtcgactctagtcaaagagggcgagataat

SEQ ID NO: 24 - DNA, 46 bp, Artificial Sequence
  Artificial Sequence
gttcatgagacacccagtaggacgacctacagaatactagtcagtg

SEQ ID NO: 25 - DNA, 46 bp, Artificial Sequence
  Artificial Sequence
cactgactagtattctgtaggtcgtcctactgggtgtctcatgaac

SEQ ID NO: 26 - DNA, 56 bp, Artificial Sequence
  Artificial Sequence
cagctatgaccatgattacgaattcgagctcggtacccaccgcacgatggttcact

SEQ ID NO: 27 - DNA, 19 bp, Artificial Sequence
  Artificial Sequence
tcaaagagggcgagataat

SEQ ID NO: 28 - DNA, 18 bp, Artificial Sequence
  Artificial Sequence
accgcacgatggttcact

SEQ ID NO: 29 - DNA, 192 bp, Corynebacterium glutamicum
cttaagtctcatatttcaaacatagttccacctgtgtgattaatccctagaacggaacaaactgatgaacaatcgttaacaacacagaccaaaacggtcagttaggtatggatatcagcaccttctgaacgggtacgtctagactggtgggcgtttgaaaaactcttcgccccacgaaaatgaaggagcata

SEQ ID NO: 30 - DNA, 192 bp, Artificial Sequence
  Artificial Sequence
cttaagtctcatatttcaaacatagttccacctgtgtgattaatccctagaacggaacaaactgatgaacaatcgttaacaacacagaccaaaacggtcagttaggtatggatatcagcaccttctgaacgggttgtggtataatggtgggcgtttgaaaaactcttcgccccacgaaaatgaaggagcata

SEQ ID NO: 31 - DNA, 29 bp, Artificial Sequence
  Artificial Sequence
ccggaattcaccatgccggacatgcggac

SEQ ID NO: 32 - DNA, 30 bp, Artificial Sequence
  Artificial Sequence
ccttctgaacgggttgtggtataatggtgg

SEQ ID NO: 33 - DNA, 30 bp, Artificial Sequence
  Artificial Sequence
ccaccattataccacaacccgttcagaagg

SEQ ID NO: 34 - DNA, 30 bp, Artificial Sequence
  Artificial Sequence
acatgcatgcgaatattgacgttgaggaag

SEQ ID NO: 35 - DNA, 20 bp, Artificial Sequence
  Artificial Sequence
agatcgtcggactcattgac

SEQ ID NO: 36 - DNA, 20 bp, Artificial Sequence
  Artificial Sequence
caaacatagttccacctgtg